European Patent Application EP 4 748 850 A1, published May 27, 2026. Title: Protein variants and a method for producing L-arginine using the same. Applicant: CJ CheilJedang Corporation. Application KR. The sequence listing filed with the application follows.

SEQUENCE LISTING (81 sequences)

SEQ ID NO: 1 - DNA, 40 bp, synthetic construct
  source 1..40: mol_type = other DNA
tgaattcgagctcggtaccccactggtgaactccttgtcc

SEQ ID NO: 2 - DNA, 40 bp, synthetic construct
  source 1..40: mol_type = other DNA
ttgaactaggggcgctttaaaagttttccggtgttgacgg

SEQ ID NO: 3 - DNA, 40 bp, synthetic construct
  source 1..40: mol_type = other DNA
ccgtcaacaccggaaaacttttaaagcgcccctagttcaa

SEQ ID NO: 4 - DNA, 40 bp, synthetic construct
  source 1..40: mol_type = other DNA
gtcgactctagaggatcccccgttgaactgcttgccagcc

SEQ ID NO: 5 - DNA, 40 bp, synthetic construct
  source 1..40: mol_type = other DNA
tgaattcgagctcggtaccctgcggctcgcacggttgctc

SEQ ID NO: 6 - DNA, 40 bp, synthetic construct
  source 1..40: mol_type = other DNA
acggtgcgcaagaagaccacgtcggcagcaaaagcagcct

SEQ ID NO: 7 - DNA, 40 bp, synthetic construct
  source 1..40: mol_type = other DNA
ggctgcttttgctgccgacgtggtcttcttgcgcaccgtg

SEQ ID NO: 8 - DNA, 40 bp, synthetic construct
  source 1..40: mol_type = other DNA
gtcgactctagaggatccccctcttatcaggccaatcggt

SEQ ID NO: 9 - DNA, 42 bp, synthetic construct
  source 1..42: mol_type = other DNA
gtgaattcgagctcggtacccgccccgaaaagccgttaaaag

SEQ ID NO: 10 - DNA, 42 bp, synthetic construct
  source 1..42: mol_type = other DNA
tgccaaaattcacgattattgctcgagtctagagacgggtta

SEQ ID NO: 11 - DNA, 42 bp, synthetic construct
  source 1..42: mol_type = other DNA
ttattggaggagatcaaaacaatgacaatcaaggttgcaatc

SEQ ID NO: 12 - DNA, 42 bp, synthetic construct
  source 1..42: mol_type = other DNA
caggtcggcgtcgcaccttaaggggatcctctagagtcgacc

SEQ ID NO: 13 - DNA, 21 bp, synthetic construct
  source 1..21: mol_type = other DNA
caataatcgtgaattttggca

SEQ ID NO: 14 - DNA, 21 bp, synthetic construct
  source 1..21: mol_type = other DNA
tgttttgatctcctccaataa

SEQ ID NO: 15 - protein, 481 aa, synthetic construct
MPKPLPPETRRKIIDFDPFAPNSPSIEEFCSRLKISRRSFYNIRNRYQQDANAALHPRSSAPITARRTYDESITSTLLSIRARLKAQGWEYGPISIRFEGISTGELTAPIPSVSTIARLLRAAGAVESNPKKRPKSSVVRFQRGQAMEMWQIDGFIYTLHDTDLTRVTIYQILDDATRFDVGTCVFPANENSVDARTVLEQAIAHFGAPHELLSDNGSAFNRMRQGYVGSLESYLATVGCLSITGKPGHPQTQGKNERSHRTLFRFLQAHQPHTLEECAHYIEQFRDHYNNRRPHQGLPNNLTPASAWEIVGCVEQQPPIDPVVLQQQADHYARRRIEKQSDVPLVRQEESVPVSKMQQTEQRRRVRRFGKKPVDPDVFTFAGNNQKVVFQGMRISVPRTMRDREFYRTVTATELGFWDAITGELELSIPLLVVAIARGKSYVNSYNIRGVWMQHPTPLWQRKRDEAEKRFKSIDPGDLLR

SEQ ID NO: 16 - protein, 64 aa, synthetic construct
MTTDIYFSHNNPHDPYAHHTTELNRDTHHLWVTLTTDSDDFDADSFTTEVIRITGYSRHEVNNG

SEQ ID NO: 17 - protein, 364 aa, synthetic construct
MANLDSVRPGVRAALRRTHTQVKGVALTRALIALAVSGALLSSMTPAVAQPQNPDDAAIAQAEENVSAGDGEVARLAGSLSSTDAEINRVELEMGALREEVNKSLVDLHDAQAIAEQARQDALAAKKDLDDSQAQIEAAQERLDEISRAAYRQNGTSKGLSGISGNGNSEDALDRQTYLRTSAEKQQAAVEELDRLRTENANKESVLRQARIVAEQREAEAVEKQVQTEAAIAANSEQLNVLTNNRTTLVAQRDEAERNLAIARAQADNLQGQRAEYEEFQQAEQARIQAEAEAQAAAEEKRRADEAAAQAAAEAQEAAQQAQAAEEAQAAQAAEAAQAQATQAAETQAAETQAAETQAAETQA

SEQ ID NO: 18 - protein, 203 aa, synthetic construct
MTQSLRDAKRESTRRALAETTYRMVRARGFDQVTIDEITTEVNVSRRTFSNYFANKEEAVAFVPVDRIRTELEKWEAPAGIDAAAAVRSVVAHLLASGLPMMLAELGRLGRRHPPFGPHSREAQWAVWDAVRERLHEVLHIDAPRDRRNLAMLLGALYGIVSTQLADLDLGDEGPGPEVFLALQESVGEVFTLFEPALRRIGQ

SEQ ID NO: 19 - protein, 481 aa, synthetic construct
MPKPLPPETRRKIIDFDPFAPNSPSIEEFCSRLKISRRSFYNIRNRYQQDANAALHPRSSAPITARRTYDESITSTLLSIRARLKAQGWEYGPISIRFEGISTGELTAPIPSVSTIARLLRAAGAVESNPKKRPKSSVVRFQRGQAMEMWQIDGFIYTLHDTDLTRVTIYQILDDATRFDVGTCVFPANENSVDARTVLEQAIAHFGAPHELLSDNGSAFNRMRQGYVGSLESYLATVGCLSITGKPGHPQTQGKNERSHRTLFRFLQAHQPHTLEECAHYIEQFRDHYNNRRPHQGLPNNLTPAAAWEIVGCVEQQPPIDPVVLQQQADHYARRRIEKQSDVPLVRQEESVPVSKMQQTEQRRRVRRFGKKPVDPDVFTFAGNNQKVVFQGMRISVPRTMRDREFYRTVTATELGFWDAITGELELSIPLLVVAIARGKSYVNSYNIRGVWMQHPTPLWQRKRDEAEKRFKSIDPGDLLR

SEQ ID NO: 20 - protein, 949 aa, synthetic construct
MADRLVVRGAREHNLKGVDIDLPRDSMVVFTGLSGSGKSSLAFDTIFAEGQRRYVESLSSYARMFLGQMDKPDVDLIDGLSPAVSIDQKSTNRNPRSTVGTITEVYDYLRLLYARAGTAHCPVCDARVERQTPQQMVDQILGMEEGLKFQILAPVVRTRKGEFVDLFADLASQGYSRVRVDGEVHQLSDPPKLEKQIKHDIDVVVDRLQVKASQKQRLTDSMETALRLADGVAVLEFVGLEEDDPNRLRRFSEKMSCPNGHALTVDELEPRAFSFNSPYGACPACDGLGVRTEVDIDLIIPDPDAPATKAVQPWNSSPNHSYFEKLIEGLAKALGFDPETPYSELTAAQKKALVYGSKEEVSVRYKNRYGRVRSWTAPFEGVMGYFDRKLEQTDSETQKDRLLGYTREVPCPTCKGARLKPEILAVRLDSGSHGALSIAGLTALSVHEAFEFLDNLTLGKREEMIAGAVLREIHARLKFLLDVGLSYLTLDRAAGTLSGGEAQRIRLATQIGSGLAGVLYVLDEPSIGLHQRDNQRLITTLEHLRDIGNTLIVVEHDEDTIRRADWLVDIGPRAGEFGGEVVYQGEPKGILDCEESLTGAYLSGRRTLGVPDTRREIDKERQLKVVGARENNLRGIDVKIPLGVLCCITGVSGSGKSTLVNQILAKVLANKLNRARQVPGRAKRVEGLEHLDKLVQVDQSPIGRTPRSNPATYTGVFDKVRNLFAETTEAKVRGYKPGRFSFNIKGGRCEACQGDGTLKIEMNFLPDVYVPCEVCDGQRYNRETLEVKYKGKNIAEVLGMPISEAADFFEPITSIHRYLATLVDVGLGYVRLGQAATTLSGGEAQRVKLAAELQKRSNGRTVYILDEPTTGLHFEDIRKLMMVIQGLVDKGNSVIIIEHNLDVIKAADWIVDMGPEGGSGGETVVAEGTPEQVAEVAGSYTGQFLKELL

SEQ ID NO: 21 - DNA, 1446 bp, synthetic construct
  source 1..1446: mol_type = other DNA
atgcctaaacccctacccccagaaacccgacgcaagatcatcgatttcgatccgttcgcaccgaacagcccctcgatcgaagagttctgcagtcggctaaaaatatcgcggcgcagcttctacaacatccgcaaccgataccaacaagacgccaacgcagcactgcatccacgctccagcgccccaatcaccgcccggcgaacgtacgatgaatccatcaccagcaccttgctgtccatccgcgcacgcctgaaagcccaaggatgggagtacggcccgatctctattcgattcgaaggcatctccaccggggaactgactgcaccgattccatctgtttcaaccattgctcgtttgttacgcgccgcaggagctgttgaaagtaaccctaagaagcgaccgaagtcgtcggtggtgaggtttcaacgaggtcaagccatggaaatgtggcaaatagatggtttcatctacacactgcacgatactgatctgactcgggtaacgatctatcaaatccttgatgatgccactcggtttgatgtcggaacctgtgtctttcccgcgaatgaaaactcagtcgatgcccgaacagtgctagaacaagccattgctcattttggtgccccgcatgaattactcagtgataacggctcagcgtttaaccggatgcggcaaggatacgtcggaagcttggaaagctatctcgcgacggtggggtgtttaagcattaccggcaagcctgggcatcctcaaacccaaggtaaaaacgaacgcagccaccgcacactatttcgtttccttcaagctcatcaaccacacacacttgaggaatgcgcgcactatattgaacagttccgcgatcattacaacaatcgtcgcccgcatcaggggttgccgaataatctcaccccggcctcggcctgggagattgtgggctgtgtggaacaacaacccccgattgatcccgtcgtgcttcaacagcaagccgatcactatgcccgtcgtcgaattgagaagcaatcagatgtcccgcttgttcggcaggaggaatctgttccggtgtctaagatgcagcagaccgagcaacgtcgacgggtacgtcgttttggtaaaaagccggtggatcctgatgtgtttacgtttgctgggaataatcagaaggtggtgttccaggggatgcgtatttctgttcctcgtacgatgagggacagggagttttatcggacggtgacggcaactgagcttggtttctgggatgcgataaccggggagcttgagttgtcgattccgttgctggttgtggcgattgcccggggtaagtcgtatgtcaattcttacaacattcgtggggtgtggatgcaacacccgacaccgttgtggcaacgcaaacgtgatgaggctgagaagcgatttaagtcgatagatccgggggatcttctgcgctag

SEQ ID NO: 22 - DNA, 1167 bp, synthetic construct
  source 1..1167: mol_type = other DNA
atgaccactgacatctacttcagccacaacaacccacacgacccatacgcccaccacaccaccgaactcaaccgcgacacccatcacctctgggtcaccctcaccaccgactccgacgacttcgacgcagactccttcaccaccgaagtcatccggatcaccggctactcccgccacgaagtcaacaacggccttaacgccatggccgcgatgaccaacctcccacacctacgcgccatccaagaacgctactacttcctgagcatccgctacctcgcctccatcatgatcgccgtggccaaagcagaccccaccctgtgggaagaactcgacctgcgcatcaccgacgccttaacaccagtcaccgcaggggaagtcatgatccaatcctccaccctggctaaacgcatcgccgcctggatcaaagaactcgaccccgaacccaccgaggaccccacaccgaaagaggactatgttcacgtccacaccaccgatgaggcgacctatgtccgcatcaaaatcagcggccccaaccgcctgctcctcaatgacatcatcacccaactcaaagacacagacaccgaggacagcctgcctgaagcgctcatggccttcctgacagagaaaatccagttaaagatcaccaaatacctcttcaccccacacaatcaccctgagcaggcatggtcaccagactacggtgacattgatcccgaagcctacgacaatgccaccctcgtgtgcgccaaggacttagatgaggtcgctggagccacggagaagagctacaccccgagtgagaagatgaaagccctgatcagagctcgggatgggcattgccgcttcccagggtgttgcgtcccggccagtaaatgccaggtcgatcacattatcccgtgggcggagggcggcccgacagcggcgtggaacctgcagttgttgtgccagcggcatcacaatatgaaaaccgatggtcgctttactgctgatgctaatggattggcggagattagatggattgggccgatggatgtaccagcggtaactaggccgacgggtccgttggtgaaagcgatgccgcgggggatttggggtcaggtgttgagggatcggatccaggctaggtttgagcggatccgcgaccgcgccctcaacaaagaagactag

SEQ ID NO: 23 - DNA, 1968 bp, synthetic construct
  source 1..1968: mol_type = other DNA
gtggccaatctagattcagttcgccctggggtgcgggcagctcttcgacgtacccatacccaggtaaaaggtgtcgcgttgaccagggcattgattgcgcttgcagtaagcggagctttgcttagttccatgactccggcggtggcgcagccacagaatccggatgacgcagccattgcacaggcagaggaaaatgtttcggcgggcgatggggaagtcgcccgcctggcaggatctttgtccagcactgacgcggaaattaaccgcgtcgagctggaaatgggtgctctgcgtgaagaagtgaacaagtccctcgtggatttgcatgatgcgcaggcaatcgccgaacaggcccgccaagatgctcttgcagccaagaaggatctcgatgattctcaagcgcagatcgaagcagcccaagagcgccttgatgagatttcacgtgcagcgtatcgccaaaacggaacctccaaggggctttccggcatttcgggcaatggaaattctgaagatgcgctagatcgtcagacttacctgcgaaccagtgcggaaaagcagcaggcagctgttgaagagcttgatcgcctccgtacggaaaacgccaacaaggaatcggtgttgcgccaggcccgcatcgttgctgagcagcgtgaggcggaagccgtcgaaaagcaagtccagaccgaggctgcaattgccgcaaacagcgagcagctcaatgtcttgactaacaaccgcactaccttggttgcccagcgtgatgaggctgagcgcaacttggccatcgctcgtgcgcaggcggataatctgcaaggtcagcgtgctgagtacgaggaattccagcaggcagagcaggctcgcatccaggcggaagcggaagctcaggctgctgcggaggagaagcgtcgtgccgatgaggctgctgcacaggcagccgctgaagctcaagaggctgcccagcaagctcaggcagcggaggaagcccaagctgcgcaagcagctgaggcagcacaggcacaagcaactcaagctgcagaaacccaagctgcagaaacccaagctgcagaaacccaagctgcagaaacccaagctgcagaaacccaagctgcagaaacccaagctgcacaagccgcgcaagctcaggcagaagcgaatgatcgtgccgccgcgcaacagcgtgctgcagaggctcaagcagcagcggaacaggcgcaacgtgaggctgacgctcaggcggccaacgatgcccaagctcaggtactgcgtgaacaggcgctcactgcagcctccatcgctgcggctgctctaattgcggcgagccagtccagccatgccactactcaaaatccttacccaactgatgaagacgcggatccgaccgatattgcggacatccaaggcccaacgcagccaggtacgggtgagtctggagattcccagaacgactccagcgacaatgattccacaggcaacgattccacaggctctgactcttcagattcagattcctccggcaacgattcttcagaggttatttccggcgatcgttccgctcagattgagactgtgattgcgcgcgccatgagccagttgggtgtgcagtacgcatggggtggcggtaacgctaatggcccaactctgggtatccgtgacggtggcgtggcggactcttacggcgattacaacaaggttggcttcgactgctctggactgaccttgtatgcgtttgcgggtgtgggaatttcacttcctcactacacgggctaccagtaccagcacggcaccaaggtgtcgccttctgagatgcaacgtggcgatctgatcttctatggtccgggagcgtctcagcacgtggcaatttacctcggtgatggtcagatgattgaggctccgaattcgggttctgtcgtgaagatttctcctgttcgctggagcggaatgaccgagagcgtggtacgcctcatttag

SEQ ID NO: 24 - DNA, 612 bp, synthetic construct
  source 1..612: mol_type = other DNA
atgacgcagagcctgagagacgccaagcgggagtcgacccggcgagcgctcgccgagaccacctaccggatggtgcgtgcccgcggtttcgaccaggtgaccatcgacgagatcaccaccgaggtcaacgtctcccgccgtaccttctccaattacttcgccaacaaagaggaggcggtcgccttcgtgccggtcgaccgcatccggacggaactggagaagtgggaggcgccggcgggcatcgacgcggcggctgccgtgcgttccgtcgtcgcccacctgctcgccagcgggctgccgatgatgctcgccgagctcggtcgcctgggccgccgtcaccccccgttcggcccccacagcagggaggcccagtgggcggtgtgggacgcggtccgggaaaggctccacgaggtgctgcacatcgatgccccccgtgaccgccgtaacctcgcgatgctgctcggcgcgctctacggcatcgtgtcgacgcagctcgctgacctggatctgggcgacgaggggccgggccccgaggtgttcctggcgctgcaggagagcgtgggggaggtgttcacgctgttcgaaccggccctgcgccggatcgggcaatga

SEQ ID NO: 25 - DNA, 1446 bp, synthetic construct
  source 1..1446: mol_type = other DNA
atgcctaaacccctacccccagaaacccgacgcaagatcatcgatttcgatccgttcgcaccgaacagcccctcgatcgaagagttctgcagtcggctaaaaatatcgcggcgcagcttctacaacatccgcaaccgataccaacaagacgccaacgcagcactgcatccacgctccagcgccccgatcaccgcccggcgaacgtacgatgaatccatcaccagcaccttgctgtccatccgcgcacgcctgaaagcccaaggatgggagtacggcccgatctctattcgattcgaaggcatctccaccggggaactgactgcaccgattccatctgtttcaaccattgctcgtttgttacgcgccgcaggagctgttgaaagtaaccctaagaagcgaccgaagtcgtcggtggtgaggtttcaacgaggtcaagccatggaaatgtggcaaatagatggtttcatctacacactgcacgatactgatctgactcgggtcacgatctatcaaatccttgatgatgccactcggtttgatgtcggaacctgtgtctttcccgcgaatgaaaactcagtcgatgcccgaacagtgctagaacaagccattgctcatttcggtgccccgcatgaattactcagtgataacggctcagcgtttaaccggatgcggcaaggatacgtcggaagcttggaaagctatctcgcgacggtggggtgtttaagcattaccggcaagcctgggcatcctcaaacccaaggtaaaaacgaacgcagccaccgcacactatttcgtttccttcaagctcatcaaccacacacacttgaggaatgtgcgcactatattgaacagttccgcgatcattacaacaatcgtcgcccgcatcaggggttgccgaataatctcaccccggccgcggcctgggagattgtgggctgtgtggaacaacaacccccgattgatcccgtcgtgcttcaacagcaagccgatcactatgcccgtcgtcgaattgagaagcaatcagatgtcccgcttgttcggcaggaggaatctgttccggtgtctaagatgcagcagaccgagcaacgtcgacgggtacgtcgttttggtaaaaagccggtggatcctgatgtgtttacgtttgctgggaataatcagaaggtggtgttccaggggatgcgtatttctgttcctcgtacgatgagggacagggagttttatcggacggtgacggcaactgagcttggtttctgggatgcgataaccggggagcttgagttgtcgattccgttgctggttgtggcgattgcccggggtaagtcgtatgtcaattcttacaacattcgtggggtgtggatgcaacacccgacaccgttgtggcaacgcaaacgtgatgaggctgagaagcgatttaagtcgatagatccgggggatcttctgcgctag

SEQ ID NO: 26 - DNA, 2850 bp, synthetic construct
  source 1..2850: mol_type = other DNA
ttggctgatcgcctcgtagtgcgcggagcgcgtgaacacaacctaaaaggcgtggatattgatctgccacgcgactcgatggtggtgttcaccggcctgtcaggttccggtaaatcatcactggcctttgacaccatctttgcggaaggccagcgccgttacgtggagtcgttgtccagttacgcccgcatgttcttggggcagatggacaagccggacgtggatttgattgatggattatccccagcggtctccattgaccaaaagtccaccaaccgcaaccctcggtccaccgtcggtaccatcacggaagtctatgactacctgcgtcttctgtatgcccgcgctggtaccgcacactgcccagtgtgtgatgcccgcgtggagcgtcaaaccccgcagcagatggtggaccagatccttggcatggaggagggactgaagttccaaatccttgcgcctgtggtgcgtacccgtaaaggtgagttcgttgatcttttcgcagatcttgcatcccaaggttattcccgcgtgcgggttgatggggaagtgcaccagctctcggatcctccaaagctagaaaagcagatcaagcacgatattgatgttgtggttgaccgtctgcaggtaaaagccagccaaaagcagcgcctgacagactctatggaaaccgcacttcgcctggccgatggcgtggctgtgctggagttcgttggcctggaggaagatgatccgaataggcttcgtcgattctctgaaaagatgagctgccctaacggtcacgcgttgacggttgatgagctggagcctcgtgctttttccttcaactctccttatggcgcgtgtcctgcctgtgatggcttgggtgtgcgcaccgaagttgatattgatctgatcatcccagatccagatgcacctgcaactaaagcggttcagccctggaactccagcccaaaccactcttactttgaaaagctcattgaaggcctggcgaaagccctcggatttgatccggaaactccgtacagtgagctcaccgcagctcaaaagaaggctctggtctatggatcgaaggaagaagtaagcgttcgatacaagaaccgctacggacgcgtgcgttcttggactgcgccttttgaaggtgtcatgggctactttgatcgcaagttggagcagactgattccgaaacccaaaaagaccgactgttgggctacacccgtgaagtgccctgcccaacctgtaaaggcgcacgcctcaagccggaaatcttggccgtacgcctagactccggaagccatggagcgttgtccattgctggactaaccgcgctgtcggtgcatgaagcattcgagtttttggataacctcacactgggcaagcgcgaggaaatgatcgcgggagctgtgctgagggaaattcacgcccgcctgaaattcttgcttgacgtgggcctttcctacctcacccttgatcgcgccgcaggcaccctgtctggtggtgaagcgcagcgtatccgcctggctactcaaattggttccggtctggctggtgtgctctacgtcttggatgagccatccattggtctgcaccaacgtgacaaccagcgcttaatcactacccttgagcatctccgagatatcggaaacacactcattgttgtggaacacgatgaagacaccatcaggcgcgcagattggctcgtggatattggtcctcgagctggtgaatttggtggtgaagtggtctaccaaggtgagccgaagggcattttggactgcgaagaatccctcacaggtgcttacttgtctggtcgtcgaaccctgggtgttcctgatactcgccgtgagatcgacaaagagcgacagctcaaggtggttggtgctagggaaaacaacctgcggggcatcgatgtgaaaatcccactgggtgtgctgtgctgcatcactggtgtgtcgggatctggtaaatccacgctggtcaatcagattttggccaaggttctggccaacaaactcaaccgcgcacgccaagtgcctggtcgcgcaaagcgggtggaaggcctcgagcacttggataagttggtccaggtggatcagtcgccaattggtcgtactccacgttcaaacccagcgacgtacacgggtgtgtttgataaagtccgtaacctttttgccgagaccactgaagcgaaggtccgcggttacaagcctggccgcttctccttcaatattaagggtggacgctgcgaagcatgtcagggcgatggcacgctgaagatcgaaatgaacttcctgcccgacgtgtatgttccgtgtgaagtctgtgatggtcagcgctacaaccgcgagaccctcgaggtgaagtacaagggcaaaaacatcgctgaagtattgggcatgccgatctctgaggctgcggacttctttgagcccatcacctcaattcaccgatacctagcaacgctggttgatgtcggccttggctatgtccgtttgggccaggcagcaacaaccttgtctggtggtgaagcccagcgtgtgaaacttgccgctgagctgcagaagcgttccaacggtcgcaccgtttacatcctcgatgagccaactactggtttgcactttgaagatattcgcaaactcatgatggtgatccaaggcctggtggacaagggtaactccgtgatcatcatcgagcacaacctcgacgtgatcaaggctgccgactggatcgtggacatgggtccagaaggcggaagcggcggtgaaactgtggtcgctgaaggaaccccagagcaagttgctgaagttgcgggttcctacaccggccaattccttaaagagttgttgtag

SEQ ID NO: 27 - DNA, 3092 bp, synthetic construct
  source 1..3092: mol_type = other DNA
tttgttgttttgtagggcacacggtggatgccttggcatatcaagccgatgaaggacgtgagaggctgcgttatgcctcggggagttgccaactaagcgttgatccgaggatgtccgaatggggaaacccagccgcagtgatgtgtggttacctgccagtgaatgtatagctggtgtggaggttgacacggggaagtgaaacatctcagtacccgtaggagaagaaaacaattgtgattccgttagtagtggcgagcgaacgtggatgatggctaaaacttatgtgtgtgatacccggcaggggttgcatgtaggtggttgtggggcaatgacgttcatattctgccggatgtgggcatgtgctgcgtggttagtggaagtggtgtggaaacacctgccgtagaaggtgagagtcctgtacacgaagatcatggtggtgtgtgtggttgttgataccccgagtagcagcgggctcgtggaatctgctgtgaattagccgggaccacccggtaagcctgaatacttgatatgaccgatagcggattagtaccgtgagggaatggtgaaaagtaccccgggaggggagtgaaatagtacctgaaaccgtgtgctgtcaatccgtcagagcacccgtttgtggtgtgatggcgtgccttttgaagaatgagcctgcgagtcagcggcatgtcgcgaggttaacccgtgtggggtagtcgtagggaaaccgaatcctaacgagggtgtttttagtggcatgtcttggacccgaagcggagtgatctacccatggccagtgtgaagcagctgtaagaggttgtggaggcgcgaacccacttaggttgaaaactgaggggatgagttgtgggtaggggtgaaaggccaatcaaactccgtgatagctggttctccccgaaatgcatttaggtgcagcgtcgtgtgtttcttgccggaggtagagctactggatggtttagcgggaccaacatcttagcgacatcagccaaactccgaatgccggtaagttagagcacggcagtgagactgcgggggataagcttcgtagtcgagagggaaacagcccagatcgccggctaaggcccctaagggtgtgctaagtggaaaaggaggtggggtcgcgaagacagccaggaggttggcttagaagcagccatccttgaaagagtgcgtaatagctcactggtcgagtgattccgcgccgacaatgtagtggggcttaagtacaccgccgaagccgcggcaatgatctttataggattgttgggtaggggagcgtcgtgcatgcgttgaagctttggggtgaccttgggtggagtgtgtgcgagtgagaatgcaggcatgagtaacgaatgatgcgtgagaaacgtatccgccggatgactaagggttcctgggtcaagttaatcttcccagggtgagtcggggcctaaggcgaggccgacaggcgtagtcgatggataacgggttgatattcccgtacccgagtatgagcgaccatggtgaatcagtgatactaaccacccataagcacccgcgaaaaggctttgcttttttgtggtgtgtggttgcgtgggacctgatctggtagtagctaagtgatggggtgacgcagggaggtagctcagccacttattggattgtggtgtaagcgtgtggcacgcagtgtaggtcaaatccgcactgtttttgtgtgaggcgtgatgcggagcccgttaagggtgaagtgggtgatcctgtgctgtcgagaaaagcctctagcgatgttgatattcggcccgtaccctaaaccgacacaggtagtcaggtagagaatactaaggcgttcgggtgaactgtggttaaggaactcggcaaaatgcccccgtaacttcgggagaaggggggccacggcgtgtgaacaacttttcgttgggagcgtgttgtggtcgcagagaatagagggaagcgactgtttactaaaaacacaggtccgtgcgaagacgtttaagttgatgtatacggactgacgcctgcccggtgctggaaggttaagaggaccggttagtgacctttatggttgcgaagctgagaatttaagccccagtaaacggcggtggtaactataaccatcctaaggtagcgaaattccttgtcgggtaagttccgacctgcacgaatggcgtaacgacttccctgctgtctcaaccacaggcccggtgaaattgcagtacgagtaaagatgctcgttacgcgcggcaggacgaaaagaccccgggaccttcactatagcttggtattggtgtttgattcggtttgtgtaggataggtgggagacttcgatcatatgacgctagttgtgtgtgagtcgttggtgaaataccactctgatcggattggatgtcttaaccttggcccatgatctgggttggggacagtgcctggtgggtagtttaactggggcggttgcctcctaaaatgtaacggaggcgcccaaaggtttcctcagcttggttggtaatcaggtggtgagtgtaagtgcacaagggagcttgactgtgacactgacaggtggagcagggacgaaagtcgggactagtgatccggcacctacttgtggttgtggtgtcgctcaacggataaaaggtaccccggggataacaggctgatcttccccaagagtccatatcgacgggatggtttggcacctcgatgtcggctcgtcgcatcctggggctggagtaggtcccaagggttgggctgttcgcccattaaagcggcacgcgagctgggtttagaacgtcgtgagacagttcggtctctatccgccgcgcgcgttgaaacttgaaggaaggctgtccctagtacgagaggaccgggacggacgtacctctggtgtgccagttgttccgccaggagcagggctggttggctacgtacgggagggataaccgctgaaagcatctaagcgggaagcctgtttcgagatgaggtttcttttgaggttccctagagattatggggttgataggccagatctggaagcactgtgaggtgtggaggtgactggtactaatttaccgataacaacaaaccac

SEQ ID NO: 28 - DNA, 3084 bp, synthetic construct
  source 1..3084: mol_type = other DNA
tttgttgttttgtagggcacacggtggatgccttggcatatcaagccgatgaaggacgtgagaggctgcgttatgcctcggggagttgccaactaagcgttgatccgaggatgtccgaatggggaaacccagccgcagtgatgtgtggttacctgccagtgaatgtatagctggtgtggaggttgacacggggaagtgaaacatctcagtacccgtaggagaagaaaacaattgtgattccgttagtagtggcgagcgaacgtggatgatggctaaaacttatgtgtgtgatacccggcaggggttgcatgtaggtggttgtggggcaatgacgttcatattctgccggatgtgggcatgtgctgcgtggttagtggaagtggtgtggaaacacctgccgtagaaggtgagagtcctgtacacgaagatcatggtggtgtgtgtggttgttgataccccgagtagcagcgggctcgtggaatctgctgtgaattagccgggaccacccggtaagcctgaatacttgatatgaccgatagcggattagtaccgtgagggaatggtgaaaagtaccccgggaggggagtgaaatagtacctgaaaccgtgtgctgtcaatccgtcagagcatccttatgtggtgtgatggcgtgccttttgaagaatgagcctgcgagtcagcggcatgtcgcgaggttaacccgtgtggggtagccgtagggaaaccgaatcctaacgagggtgattttagtggcatgtcttggacccgaagcggagtgatctacccatggccagtgtgaagcagctgtaagaggttgtggaggcgcgaacccacttaggttgaaaactgaggggatgagttgtgggtaggggtgaaaggccaatcaaactccgtgatagctggttctccccgaaatgcatttaggtgcagcgtcgtgtgtttcttgccggaggtagagctactggatggtttagcgggaccaacatcttagcgacatcagccaaactccgaatgccggtaagtcagagcacggcagtgagactgcgggggataagcttcgtagtcgagagggaaacagcccagatcgccggctaaggcccctaagggtgtgctaagtggaaaaggaggtggggtcgcgaagacagccaggaggttggcttagaagcagccatccttgaaagagtgcgtaatagctcactggtcgagtgattccgcgccgacaatgtagtggggcttaagtacaccgccgaagccgcggcaatgatctttattggattgttgggtaggggagcgtcgtgcatgcgttgaagctttggggtgaccttgggtggagtgtgtgcgagtgagaatgcaggcatgagtaacgaatgatgcgtgagaaacgtatccgccggatgactaagggttcctgggtcaagttaatcttcccagggtgagtcggggcctaaggcgaggccgacaggcgtagtcgatggataacgggttgatattcccgtacccgagtatgagcgaccatggtgaatcagtgatactaaccacccataagcacccgcgaaaaggctttgcttttttgtggtgtgtggttgcgtgggacctgatctggtagtagctaagtgatggggtgacgcagggaggtagctcagccacttattggattgtggtgtaagcgtgtggcacgcagtgtaggtcaaatccgcactgtttttgtgtgaggcgtgatgcggagcccgtaaagggtgaagtgggtgatcctgtgctgtcgagaaaagcctctagcgatgttgatattcggcccgtaccctaaaccgacacaggtagtcaggtagagaatactaaggcgttcgggtgaactgtggttaaggaactcggcaaaatgcccccgtaacttcgggagaaggggggccacggcgtgtgaacaacttttcgttgggagcgtgttgtggtcgcagagaatagagggaagcgactgtttactaaaaacacaggtccgtgcgaagacgtttaagttgatgtatacggactgacgcctgcccggtgctggaaggttaagaggaccggttagccgtaaggcgaagctgagaatttaagccccagtaaacggcggtggtaactataaccatcctaaggtagcgaaattccttgtcgggtaagttccgacctgcacgaatggcgtaacgacttccctgctgtctcaaccacaggcccggtgaaattgcagtacgagtaaagatgctcgttacgcgcggcaggacgaaaagaccccgggaccttcactatagcttggtattggtgtttgattcggtttgtgtaggataggtgggagacttcgatcatatgacgctagttgtgtgtgagtcgttggtgaaataccactctgatcggattggatgtcttaaccttggcccatgatctgggttggggacagtgcctggtgggtagtttaactggggcggttgcctcctaaaatgtaacggaggcgcccaaaggtttcctcagcttggttggtaatcaggtggtgagtgtaagtgcacaagggagcttgactgtgacactgacaggtggagcagggacgaaagtcgggactagtgatccggcacctacttgtggttgtggtgtcgctcaacggataaaaggtaccccggggataacaggctgatcttccccaagagtccatatcgacgggatggtttggcacctcgatgtcggctcgtcgcatcctggggctggagtaggtcccaagggttgggctgttcgcccattaaagcggcacgcgagctgggtttagaacgtcgtgagacagttcggtctctatccgccgcgcgcgttgaaacttgaaggaaggctgtccctagtacgagaggaccgggacggacgtacctctggtgtgccagttgttccgccaggagcagggctggttggctacgtacgggagggataaccgctgaaagcatctaagcgggaagcctgtttcgagatgaggtttcttttgaggttccctagagattatggggttgataggccagatctggaagcactgtgaggtgtggaggtgactggtactaatttaccgataacaacaaacca

SEQ ID NO: 29 - DNA, 3091 bp, synthetic construct
  source 1..3091: mol_type = other DNA
tttgttgttttgtagggcacacggtggatgccttggcatatcaagccgatgaaggacgtgagaggctgcgttatgcctcggggagttgccaactaagcgttgatccgaggatgtccgaatggggaaacccagccgcagtgatgtgtggttacctgccagtgaatgtatagctggtgtggaggttgacacggggaagtgaaacatctcagtacccgtaggagaagaaaacaattgtgattccgttagtagtggcgagcgaacgtggatgatggctaaaacttatgtgtgtgatacccggcaggggttgcatgtaggtggttgtggggcaatgacgttcatattctgccggatgtgggcatgtgctgcgtggttagtggaagtggtgtggaaacacctgccgtagaaggtgagagtcctgtacacgaagatcatggtggtgtgtgtggttgttgataccccgagtagcagcgggctcgtggaatctgctgtgaattagccgggaccacccggtaagcctgaatacttgatatgaccgatagcggattagtaccgtgagggaatggtgaaaagtaccccgggaggggagtgaaatagtacctgaaaccgtgtgctgtcaatccgtcagagcacccctttgtggtgtgatggcgtgccttttgaagaatgagcctgcgagtcagcggcatgtcgcgaggttaacccgtgtggggtagccgtagggaaaccgaatcctaacgagggtgattttagtggcatgtcttggacccgaagcggagtgatctacccatggccagtgtgaagcagctgtaagaggttgtggaggcgcgaacccacttaggttgaaaactgaggggatgagttgtgggtaggggtgaaaggccaatcaaactccgtgatagctggttctccccgaaatgcatttaggtgcagcgtcgtgtgtttcttgccggaggtagagctactggatggtttagcgggaccaacatcttagcgacatcagccaaactccgaatgccggtaagtcagagcacggcagtgagactgcgggggataagcttcgtagtcgagagggaaacagcccagatcgccggctaaggcccctaagggtgtgctaagtggaaaaggaggtggggtcgcgaagacagccaggaggttggcttagaagcagccatccttgaaagagtgcgtaatagctcactggtcgagtgattccgcgccgacaatgtagtggggcttaagtacaccgccgaagccgcggcaatgatctttataggattgttgggtaggggagcgtcgtgcatgcgttgaagctttggggtgaccttgggtggagtgtgtgcgagtgagaatgcaggcatgagtaacgaatgatgcgtgagaaacgtatccgccggatgactaagggttcctgggtcaagttaatcttcccagggtgagtcggggcctaaggcgaggccgacaggcgtagtcgatggataacgggttgatattcccgtacccgagtatgagcgaccatggtgaatcagtgatactaaccacccataagcacccgcgaaaaggctttgcttttttgtggtgtgtggttgcgtgggacctgatctggtagtagctaagtgatggggtgacgcagggaggtagctcagccacttattggattgtggtgtaagcgtgtggcacgcagtgtaggtcaaatccgcactgtttttgtgtgaggcgtgatgcggagcccgttaagggtgaagtgggtgatcctgtgctgtcgagaaaagcctctagcgatgttgatattcggcccgtaccctaaaccgacacaggtagtcaggtagagaatactaaggcgttcgggtgaactgtggttaaggaactcggcaaaatgcccccgtaacttcgggagaaggggggccacggcgtgtgaacaacttttcgttgggagcgtgttgtggtcgcagagaatagagggaagcgactgtttactaaaaacacaggtccgtgcgaagacgtttaagttgatgtatacggactgacgcctgcccggtgctggaaggttaagaggaccggttagtgacctttatggttgcgaagctgagaatttaagccccagtaaacggcggtggtaactataaccatcctaaggtagcgaaattccttgtcgggtaagttccgacctgcacgaatggcgtaacgacttccctgctgtctcaaccacaggcccggtgaaattgcagtacgagtaaagatgctcgttacgcgcggcaggacgaaaagaccccgggaccttcactatagcttggtattggtgtttgattcggtttgtgtaggataggtgggagacttcgatcatatgacgctagttgtgtgtgagtcgttggtgaaataccactctgatcggattggatgtcttaaccttggcccatgatctgggttggggacagtgcctggtgggtagtttaactggggcggttgcctcctaaaatgtaacggaggcgcccaaaggtttcctcagcttggttggtaatcaggtggtgagtgtaagtgcacaagggagcttgactgtgacactgacaggtggagcagggacgaaagtcgggactagtgatccggcacctacttgtggttgtggtgtcgctcaacggataaaaggtaccccggggataacaggctgatcttccccaagagtccatatcgacgggatggtttggcacctcgatgtcggctcgtcgcatcctggggctggagtaggtcccaagggttgggctgttcgcccattaaagcggcacgcgagctgggtttagaacgtcgtgagacagttcggtctctatccgccgcgcgcgttgaaacttgaaggaaggctgtccctagtacgagaggaccgggacggacgtacctctggtgtgccagttgttccgccaggagcagggctggttggctacgtacgggagggataaccgctgaaagcatctaagcgggaagcctgtttcgagatgaggtttcttttgaggttccctagagattatggggttgataggccagatctggaagcactgtgaggtgtggaggtgactggtactaatttaccgataacaacaaacca

SEQ ID NO: 30 - DNA, 3092 bp, synthetic construct
  source 1..3092: mol_type = other DNA
tttgttgttttgtagggcacacggtggatgccttggcatatcaagccgatgaaggacgtgagaggctgcgttatgcctcggggagttgccaactaagcgttgatccgaggatgtccgaatggggaaacccagccgcagtgatgtgtggttacctgccagtgaatgtatagctggtgtggaggttgacacggggaagtgaaacatctcagtacccgtaggagaagaaaacaattgtgattccgttagtagtggcgagcgaacgtggatgatggctaaaacttatgtgtgtgatacccggcaggggttgcatgtaggtggttgtggggcaatgacgttcatattctgccggatgtgggcatgtgctgcgtggttagtggaagtggtgtggaaacacctgccgtagaaggtgagagtcctgtacacgaagatcatggtggtgtgtgtggttgttgataccccgagtagcagcgggctcgtggaatctgctgtgaattagccgggaccacccggtaagcctgaatacttgatatgaccgatagcggattagtaccgtgagggaatggtgaaaagtaccccgggaggggagtgaaatagtacctgaaaccgtgtgctgtcaatccgtcagagcacccgtttgtggtgtgatggcgtgccttttgaagaatgagcctgcgagtcagcggcatgtcgcgaggttaacccgtgtggggtagccgtagggaaaccgaatcctaacgagggtgtttttagtggcatgtcttggacccgaagcggagtgatctacccatggccagtgtgaagcagctgtaagaggttgtggaggcgcgaacccacttaggttgaaaactgaggggatgagttgtgggtaggggtgaaaggccaatcaaactccgtgatagctggttctccccgaaatgcatttaggtgcagcgtcgtgtgtttcttgccggaggtagagctactggatggtttagcgggaccaacatcttagcgacatcagccaaactccgaatgccggtaagtcagagcacggcagtgagactgcgggggataagcttcgtagtcgagagggaaacagcccagatcgccggctaaggcccctaagggtgtgctaagtggaaaaggaggtggggtcgcgaagacagccaggaggttggcttagaagcagccatccttgaaagagtgcgtaatagctcactggtcgagtgattccgcgccgacaatgtagtggggcttaagtacaccgccgaagccgcggcaatgatctttataggattgttgggtaggggagcgtcgtgcatgcgttgaagctttggggtgaccttgggtggagtgtgtgcgagtgagaatgcaggcatgagtaacgaatgatgcgtgagaaacgtatccgccggatgactaagggttcctgggtcaagttaatcttcccagggtgagtcggggcctaaggcgaggccgacaggcgtagtcgatggataacgggttgatattcccgtacccgagtatgagcgaccatggtgaatcagtgatactaaccacccataagcacccgcgaaaaggctttgcttttttgtggtgtgtggttgcgtgggacctgatctggtagtagctaagtgatggggtgacgcagggaggtagctcagccacttattggattgtggtgtaagcgtgtggcacgcagtgtaggtcaaatccgcactgtttttgtgtgaggcgtgatgcggagcccgttaagggtgaagtgggtgatcctgtgctgtcgagaaaagcctctagcgatgttgatattcggcccgtaccctaaaccgacacaggtagtcaggtagagaatactaaggcgttcgggtgaactgtggttaaggaactcggcaaaatgcccccgtaacttcgggagaaggggggccacggcgtgtgaacaacttttcgttgggagcgtgttgtggtcgcagagaatagagggaagcgactgtttactaaaaacacaggtccgtgcgaagacgtttaagttgatgtatacggactgacgcctgcccggtgctggaaggttaagaggaccggttagtgacctttatggttgcgaagctgagaatttaagccccagtaaacggcggtggtaactataaccatcctaaggtagcgaaattccttgtcgggtaagttccgacctgcacgaatggcgtaacgacttccctgctgtctcaaccacaggcccggtgaaattgcagtacgagtaaagatgctcgttacgcgcggcaggacgaaaagaccccgggaccttcactatagcttggtattggtgtttgattcggtttgtgtaggataggtgggagacttcgatcatatgacgctagttgtgtgtgagtcgttggtgaaataccactctgatcggattggatgtcttaaccttggcccatgatctgggttggggacagtgcctggtgggtagtttaactggggcggttgcctcctaaaatgtaacggaggcgcccaaaggtttcctcagcttggttggtaatcaggtggtgagtgtaagtgcacaagggagcttgactgtgacactgacaggtggagcagggacgaaagtcgggactagtgatccggcacctacttgtggttgtggtgtcgctcaacggataaaaggtaccccggggataacaggctgatcttccccaagagtccatatcgacgggatggtttggcacctcgatgtcggctcgtcgcatcctggggctggagtaggtcccaagggttgggctgttcgcccattaaagcggcacgcgagctgggtttagaacgtcgtgagacagttcggtctctatccgccgcgcgcgttgaaacttgaaggaaggctgtccctagtacgagaggaccgggacggacgtacctctggtgtgccagttgttccgccaggagcagggctggttggctacgtacgggagggataaccgctgaaagcatctaagcgggaagcctgtttcgagatgaggtttcttttgaggttccctagagattatggggttgataggccagatctggaagcactgtgaggtgtggaggtgactggtactaatttaccgataacaacaaaccac

SEQ ID NO: 31 - DNA, 3086 bp, synthetic construct
  source 1..3086: mol_type = other DNA
tttgttgttttgtagggcacacggtggatgccttggcatatcaagccgatgaaggacgtgagaggctgcgttatgcctcggggagttgccaactaagcgttgatccgaggatgtccgaatggggaaacccagccgcagtgatgtgtggttacctgccagtgaatgtatagctggtgtggaggttgacacggggaagtgaaacatctcagtacccgtaggagaagaaaacaattgtgattccgttagtagtggcgagcgaacgtggatgatggctaaaacttatgtgtgtgatacccggcaggggttgcatgtaggtggttgtggggcaatgacgttcatattctgccggatgtgggcatgtgctgcgtggttagtggaagtggtgtggaaacacctgccgtagaaggtgagagtcctgtacacgaagatcatggtggtgtgtgtggttgttgataccccgagtagcagcgggctcgtggaatctgctgtgaattagccgggaccacccggtaagcctgaatacttgatatgaccgatagcggattagtaccgtgagggaatggtgaaaagtaccccgggaggggagtgaaatagtacctgaaaccgtgtgctgtcaatccgtcagagcacccctttgtggtgtgatggcgtgccttttgaagaatgagcctgcgagtcagcggcatgtcgcgaggttaacccgtgtggggtagccgtagggaaaccgaatcctaacgagggtgattttagtggcatgtcttggacccgaagcggagtgatctacccatggccagtgtgaagcagctgtaagaggttgtggaggcgcgaacccacttaggttgaaaactgaggggatgagttgtgggtaggggtgaaaggccaatcaaactccgtgatagctggttctccccgaaatgcatttaggtgcagcgtcgtgtgtttcttgccggaggtagagctactggatggtttagcgggaccaacatcttagcgacatcagccaaactccgaatgccggtaagtcagagcacggcagtgagactgcgggggataagcttcgtagtcgagagggaaacagcccagatcgccggctaaggcccctaagggtgtgctaagtggaaaaggaggtggggtcgcgaagacagccaggaggttggcttagaagcagccatccttgaaagagtgcgtaatagctcactggtcgagtgattccgcgccgacaatgtagtggggcttaagtacaccgccgaagccgcggcaatgatctttataggattgttgggtaggggagcgtcgtgcatgcgttgaagctttggggtgaccttgggtggagtgtgtgcgagtgagaatgcaggcatgagtaacgaatgatgcgtgagaaacgtatccgccggatgactaagggttcctgggtcaagttaatcttcccagggtgagtcggggcctaaggcgaggccgacaggcgtagtcgatggataacgggttgatattcccgtacccgagtatgagcgaccatggtgaatcagtgatactaaccacccataagcacccgcgaaaaggctttgctttttttgtggtgtgtggttgcgtgggacctgatctggtagtagctaagtgatggggtgacgcagggaggtagctcagccacttattggattgtggtgtaagcgtgtggcacgcagtgtaggtcaaatccgcactgtttttgtgtgaggcgtgatgcggagcccgttaagggtgaagtgggtgatcctgtgctgtcgagaaaagcctctagcgatgttgatattcggcccgtaccctaaaccgacacaggtagtcaggtagagaatactaaggcgttcgggtgaactgtggttaaggaactcggcaaaatgcccccgtaacttcgggagaaggggggccacggcgtgtgaacaacttttcgttgggagcgtgttgtggtcgcagagaatagagggaagcgactgtttactaaaaacacaggtccgtgcgaagacgtttaagttgatgtatacggactgacgcctgcccggtgctggaaggttaagaggaccggttagccgtaaggcgaagctgagaatttaagccccagtaaacggcggtggtaactataaccatcctaaggtagcgaaattccttgtcgggtaagttccgacctgcacgaatggcgtaacgacttccctgctgtctcaaccacaggcccggtgaaattgcagtacgagtaaagatgctcgttacgcgcggcaggacgaaaagaccccgggaccttcactatagcttggtattggtgtttgattcggtttgtgtaggataggtgggagacttcgatcatatgacgctagttgtgtgtgagtcgttggtgaaataccactctgatcggattggatgtcttaaccttggcccatgatctgggttggggacagtgcctggtgggtagtttaactggggcggttgcctcctaaaatgtaacggaggcgcccaaaggtttcctcagcttggttggtaatcaggtggtgagtgtaagtgcacaagggagcttgactgtgacactgacaggtggagcagggacgaaagtcgggactagtgatccggcacctacttgtggttgtggtgtcgctcaacggataaaaggtaccccggggataacaggctgatcttccccaagagtccatatcgacgggatggtttggcacctcgatgtcggctcgtcgcatcctggggctggagtaggtcccaagggttgggctgttcgcccattaaagcggcacgcgagctgggtttagaacgtcgtgagacagttcggtctctatccgccgcgcgcgttgaaacttgaaggaaggctgtccctagtacgagaggaccgggacggacgtacctctggtgtgccagttgttccgccaggagcagggctggttggctacgtacgggagggataaccgctgaaagcatctaagcgggaagcctgtttcgagatgaggtttcttttgaggttccctagagattatggggttgataggccagatctggaagcactgtgaggtgtggaggtgactggtactaatttaccgataacaacaaaccac

SEQ ID NO: 32 - DNA, 3093 bp, synthetic construct
  source 1..3093: mol_type = other DNA
tttgttgttttgtagggcacacggtggatgccttggcatatcaagccgatgaaggacgtgagaggctgcgttatgcctcggggagttgccaactaagcgttgatccgaggatgtccgaatggggaaacccagccgcagtgatgtgtggttacctgccagtgaatgtatagctggtgtggaggttgacacggggaagtgaaacatctcagtacccgtaggagaagaaaacaattgtgattccgttagtagtggcgagcgaacgtggatgatggctaaaacttatgtgtgtgatacccggcaggggttgcatgtaggtggttgtggggcaatgacgttcatattctgccggatgtgggcatgtgctgcgtggttagtggaagtggtgtggaaacacctgccgtagaaggtgagagtcctgtacacgaagatcatggtggtgtgtgtggttgttgataccccgagtagcagcgggctcgtggaatctgctgtgaattagccgggaccacccggtaagcctgaatacttgatatgaccgatagcggattagtaccgtgagggaatggtgaaaagtaccccgggaggggagtgaaatagtacctgaaaccgtgtgctgtcaatccgtcagagcacccctttgtggtgtgatggcgtgccttttgaagaatgagcctgcgagtcagcggcatgtcgcgaggttaacccgtgtggggtagccgtagggaaaccgaatcctaacgagggtgattttagtggcatgtcttggacccgaagcggagtgatctacccatggccagtgtgaagcagctgtaagaggttgtggaggcgcgaacccacttaggttgaaaactgaggggatgagttgtgggtaggggtgaaaggccaatcaaactccgtgatagctggttctccccgaaatgcatttaggtgcagcgtcgtgtgtttcttgccggaggtagagctactggatggtttagcgggaccaacatcttagcgacatcagccaaactccgaatgccggtaagtcagagcacggcagtgagactgcgggggataagcttcgtagtcgagagggaaacagcccagatcgccggctaaggcccctaagggtgtgctaagtggaaaaggaggtggggtcgcgaagacagccaggaggttggcttagaagcagccatccttgaaagagtgcgtaatagctcactggtcgagtgattccgcgccgacaatgtagtggggcttaagtacaccgccgaagccgcggcaatgatctttataggattgttgggtaggggagcgtcgtgcatgcgttgaagctttggggtgaccttgggtggagtgtgtgcgagtgagaatgcaggcatgagtaacgaatgatgcgtgagaaacgtatccgccggatgactaagggttcctgggtcaagttaatcttcccagggtgagtcggggcctaaggcgaggccgacaggcgtagtcgatggataacgggttgatattcccgtacccgagtatgagcgaccatggtgaatcagtgatactaaccacccataagcacccgcgaaaaggctttgctttttttgtggtgtgtggttgcgtgggacctgatctggtagtagctaagtgatggggtgacgcagggaggtagctcagccacttattggattgtggtgtaagcgtgtggcacgcagtgtaggtcaaatccgcactgtttttgtgtgaggcgtgatgcggagcccgttaagggtgaagtgggtgatcctgtgctgtcgagaaaagcctctagcgatgttgatattcggcccgtaccctaaaccgacacaggtagtcaggtagagaatactaaggcgttcgggtgaactgtggttaaggaactcggcaaaatgcccccgtaacttcgggagaaggggggccacggcgtgtgaacaacttttcgttgggagcgtgttgtggtcgcagagaatagagggaagcgactgtttactaaaaacacaggtccgtgcgaagacgtttaagttgatgtatacggactgacgcctgcccggtgctggaaggttaagaggaccggttagtgacctttatggttgcgaagctgagaatttaagccccagtaaacggcggtggtaactataaccatcctaaggtagcgaaattccttgtcgggtaagttccgacctgcacgaatggcgtaacgacttccctgctgtctcaaccacaggcccggtgaaattgcagtacgagtaaagatgctcgttacgcgcggcaggacgaaaagaccccgggaccttcactatagcttggtattggtgtttgattcggtttgtgtaggataggtgggagacttcgatcatatgacgctagttgtgtgtgagtcgttggtgaaataccactctgatcggattggatgtcttaaccttggcccatgatctgggttggggacagtgcctggtgggtagtttaactggggcggttgcctcctaaaatgtaacggaggcgcccaaaggtttcctcagcttggttggtaatcaggtggtgagtgtaagtgcacaagggagcttgactgtgacactgacaggtggagcagggacgaaagtcgggactagtgatccggcacctacttgtggttgtggtgtcgctcaacggataaaaggtaccccggggataacaggctgatcttccccaagagtccatatcgacgggatggtttggcacctcgatgtcggctcgtcgcatcctggggctggagtaggtcccaagggttgggctgttcgcccattaaagcggcacgcgagctgggtttagaacgtcgtgagacagttcggtctctatccgccgcgcgcgttgaaacttgaaggaaggctgtccctagtacgagaggaccgggacggacgtacctctggtgtgccagttgttccgccaggagcagggctggttggctacgtacgggagggataaccgctgaaagcatctaagcgggaagcctgtttcgagatgaggtttcttttgaggttccctagagattatggggttgataggccagatctggaagcactgtgaggtgtggaggtgactggtactaatttaccgataacaacaaaccac

SEQ ID NO: 33 - DNA, 40 bp, synthetic construct
  source 1..40: mol_type = other DNA
tgaattcgagctcggtaccctgaaaactcagtcgatgccc

SEQ ID NO: 34 - DNA, 40 bp, synthetic construct
  source 1..40: mol_type = other DNA
gtcgactctagaggatccccgttatcgcatcccagaaacc

SEQ ID NO: 35 - DNA, 40 bp, synthetic construct
  source 1..40: mol_type = other DNA
tgaattcgagctcggtacccggaccctgtctaaacttcgt

SEQ ID NO: 36 - DNA, 40 bp, synthetic construct
  source 1..40: mol_type = other DNA
gtcgactctagaggatcccctcaccaacggacccgtcggc

SEQ ID NO: 37 - DNA, 40 bp, synthetic construct
  source 1..40: mol_type = other DNA
tgaattcgagctcggtaccccggatccgcgtcttcatcag

SEQ ID NO: 38 - DNA, 40 bp, synthetic construct
  source 1..40: mol_type = other DNA
gtcgactctagaggatcccccagaccgaggctgcaattgc

SEQ ID NO: 39 - DNA, 40 bp, synthetic construct
  source 1..40: mol_type = other DNA
tgaattcgagctcggtacccccggggtcattgcccgatcc

SEQ ID NO: 40 - DNA, 40 bp, synthetic construct
  source 1..40: mol_type = other DNA
gtcgactctagaggatccccgacgccaagcgggagtcgac

SEQ ID NO: 41 - DNA, 40 bp, synthetic construct
  source 1..40: mol_type = other DNA
tgaattcgagctcggtaccctgtggaacaacaacccccga

SEQ ID NO: 42 - DNA, 40 bp, synthetic construct
  source 1..40: mol_type = other DNA
gtcgactctagaggatccccgcacttaatgatccgaatct

SEQ ID NO: 43 - DNA, 40 bp, synthetic construct
  source 1..40: mol_type = other DNA
tgaattcgagctcggtacccgcggacttctttgagcccat

SEQ ID NO: 44 - DNA, 40 bp, synthetic construct
  source 1..40: mol_type = other DNA
gtcgactctagaggatccccacgcgcccggcgccctttgg

SEQ ID NO: 45 - DNA, 40 bp, synthetic construct
  source 1..40: mol_type = other DNA
tgaattcgagctcggtacccacgcatgcacgacgctcccc

SEQ ID NO: 46 - DNA, 40 bp, synthetic construct
  source 1..40: mol_type = other DNA
gtcgactctagaggatcccccatgtgctgcgtggttagtg

SEQ ID NO: 47 - DNA, 40 bp, synthetic construct
  source 1..40: mol_type = other DNA
tgaattcgagctcggtaccccttatgtgtgtgatacccgg

SEQ ID NO: 48 - DNA, 40 bp, synthetic construct
  source 1..40: mol_type = other DNA
gtcgactctagaggatccccctcagcttcgccttacggct

SEQ ID NO: 49 - DNA, 40 bp, synthetic construct
  source 1..40: mol_type = other DNA
tgaattcgagctcggtacccacaatgtagtggggcttaag

SEQ ID NO: 50 - DNA, 40 bp, synthetic construct
  source 1..40: mol_type = other DNA
gtcgactctagaggatccccttgttcacacgccgtggccc

SEQ ID NO: 51 - DNA, 18 bp, synthetic construct
  source 1..18: mol_type = other DNA
gttacgcgccgcaggagc

SEQ ID NO: 52 - DNA, 18 bp, synthetic construct
  source 1..18: mol_type = other DNA
agcagtgtgcacaccaac

SEQ ID NO: 53 - DNA, 18 bp, synthetic construct
  source 1..18: mol_type = other DNA
tgcgagccaggtggtcgc

SEQ ID NO: 54 - DNA, 18 bp, synthetic construct
  source 1..18: mol_type = other DNA
cgggctcaaacggcctca

SEQ ID NO: 55 - DNA, 18 bp, synthetic construct
  source 1..18: mol_type = other DNA
caactggctcatggcgcg

SEQ ID NO: 56 - DNA, 18 bp, synthetic construct
  source 1..18: mol_type = other DNA
gatctcgatgattctcaa

SEQ ID NO: 57 - DNA, 18 bp, synthetic construct
  source 1..18: mol_type = other DNA
caccgggaagtactttac

SEQ ID NO: 58 - DNA, 18 bp, synthetic construct
  source 1..18: mol_type = other DNA
tctggcggtgggcatcct

SEQ ID NO: 59 - DNA, 18 bp, synthetic construct
  source 1..18: mol_type = other DNA
aagctatctcgcgacggt

SEQ ID NO: 60 - DNA, 18 bp, synthetic construct
  source 1..18: mol_type = other DNA
ctaccgctggaccgagtc

SEQ ID NO: 61 - DNA, 18 bp, synthetic construct
  source 1..18: mol_type = other DNA
cggttacaagcctggccg

SEQ ID NO: 62 - DNA, 18 bp, synthetic construct
  source 1..18: mol_type = other DNA
agcattgctgatcttggt

SEQ ID NO: 63 - DNA, 18 bp, synthetic construct
  source 1..18: mol_type = other DNA
aagccttttcgcgggtgc

SEQ ID NO: 64 - DNA, 18 bp, synthetic construct
  source 1..18: mol_type = other DNA
agtgaatgtatagctggt

SEQ ID NO: 65 - DNA, 18 bp, synthetic construct
  source 1..18: mol_type = other DNA
gtcaacacgggtagagaa

SEQ ID NO: 66 - DNA, 18 bp, synthetic construct
  source 1..18: mol_type = other DNA
tcaccaacgactcacaca

SEQ ID NO: 67 - DNA, 18 bp, synthetic construct
  source 1..18: mol_type = other DNA
tgtgtttcttgccggagg

SEQ ID NO: 68 - DNA, 18 bp, synthetic construct
  source 1..18: mol_type = other DNA
ggaagtcgttacgccatt

SEQ ID NO: 69 - protein, 481 aa, synthetic construct; identical to SEQ ID NO: 19

SEQ ID NO: 70 - protein, 370 aa, synthetic construct
  source 1..370: note = X residue is deleted
MTTDIYFSHNNPHDPYAHHTTELNRDTHHLWVTLTTDSDDFDADSFTTEVIRITGYSRHEVNNGPXRHGRDDHLPHLRASRRYYSXASLLAHHDRVQSRPTLWETRLRITTLHSHAGVMIILHPANASPLDQELEPTTRTHTEETRSRHTTDEPTRSHQISAHACSSXHHHHSRHRHEDSCXSAHGLPDRENPVKDHQIPLHPTQSPEQAWSPDYGDIDPEATTMPPSCAPRTXMRSLEPRRRATPRVRRXKPXSELGMGIAASQGVASRPVNARSITLSRGRRAARQRRGTCSCCASGITIXKPMVALLLMLMDWRRLDGLGRWMYQRXLGRRVRWXKRCRGGFGVRCXGIGSRLGLSGSATAPSTKKT

SEQ ID NO: 71 - protein, 645 aa, synthetic construct
MANLDSVRPGVRAALRRTHTQVKGVALTRALIALAVSGALLSSMTPAVAQPQNPDDAAIAQAEENVSAGDGEVARLAGSLSSTDAEINRVELEMGALREEVNKSLVDLHDAQAIAEQARQDALAAKKDLDDSQAQIEAAQERLDEISRAAYRQNGTSKGLSGISGNGNSEDALDRQTYLRTSAEKQQAAVEELDRLRTENANKESVLRQARIVAEQREAEAVEKQVQTEAAIAANSEQLNVLTNNRTTLVAQRDEAERNLAIARAQADNLQGQRAEYEEFQQAEQARIQAEAEAQAAAEEKRRADEAAAQAAAEAQEAAQQAQAAEEAQAAQAAEAAQAQATQAAETQAAETQAAETQAAETQAAQAAQAQAEANDRAAAQQRAAEAQAAAEQAQREADAQAANDAQAQVLREQALTAASIAAAALIAASQSSHATTQNPYPTDEDADPTDIADIQGPTQPGTGESGDSQNDSSDNDSTGNDSTGSDSSDSDSSGNDSSEVISGDRSAQIETVIARAMSQLGVQYAWGGGNANGPTLGIRDGGVADSYGDYNKVGFDCSGLTLYAFAGVGISLPHYTGYQYQHGTKVSPSEMQRGDLIFYGPGASQHVAIYLGDGQMIEAPNSGSVVKISPVRWSGMTESVVRLI

SEQ ID NO: 72 - protein, 203 aa, synthetic construct
MTQSLRDAKRESTRRALAETTYRMVRARGFDQVTIDEITTEVNVSRRTFSNYFANKEEAVAFVPVDRIRTELEKWEAPAGIDAAAAVRSVVAHLLASGLPMMLAELGRLGRRHPPFGPHSREVQWAVWDAVRERLHEVLHIDAPRDRRNLAMLLGALYGIVSTQLADLDLGDEGPGPEVFLALQESVGEVFTLFEPALRRIGQ

SEQ ID NO: 73 - protein, 481 aa, synthetic construct
MPKPLPPETRRKIIDFDPFAPNSPSIEEFCSRLKISRRSFYNIRNRYQQDANAALHPRSSAPITARRTYDESITSTLLSIRARLKAQGWEYGPISIRFEGISTGELTAPIPSVSTIARLLRAAGAVESNPKKRPKSSVVRFQRGQAMEMWQIDGFIYTLHDTDLTRVTIYQILDDATRFDVGTCVFPANENSVDARTVLEQAIAHFGAPHELLSDNGSAFNRMRQGYVGSLESYLATVGCLSITGKPGHPQTQGKNERSHRTLFRFLQAHQPHTLEECAHYIEQFRDHYNNRRPHQGLPNNLTPAAAWEIVGCVEQQPPIDPVVLQQQADHYARRRIEKQSDVPLVRQEESVPVSKMQQTEQRRRVRRFGKKPVDPDVFTFAGNNQKVVFQGMRISVPRTMRDREFYRTVTATELGFWDAITGELELSIPLPVVAIARGKSYVNSYNIRGVWMQHPTPLWQRKRDEAEKRFKSIDPGDLLR

SEQ ID NO: 74 - protein, 949 aa, synthetic construct
MADRLVVRGAREHNLKGVDIDLPRDSMVVFTGLSGSGKSSLAFDTIFAEGQRRYVESLSSYARMFLGQMDKPDVDLIDGLSPAVSIDQKSTNRNPRSTVGTITEVYDYLRLLYARAGTAHCPVCDARVERQTPQQMVDQILGMEEGLKFQILAPVVRTRKGEFVDLFADLASQGYSRVRVDGEVHQLSDPPKLEKQIKHDIDVVVDRLQVKASQKQRLTDSMETALRLADGVAVLEFVGLEEDDPNRLRRFSEKMSCPNGHALTVDELEPRAFSFNSPYGACPACDGLGVRTEVDIDLIIPDPDAPATKAVQPWNSSPNHSYFEKLIEGLAKALGFDPETPYSELTAAQKKALVYGSKEEVSVRYKNRYGRVRSWTAPFEGVMGYFDRKLEQTDSETQKDRLLGYTREVPCPTCKGARLKPEILAVRLDSGSHGALSIAGLTALSVHEAFEFLDNLTLGKREEMIAGAVLREIHARLKFLLDVGLSYLTLDRAAGTLSGGEAQRIRLATQIGSGLAGVLYVLDEPSIGLHQRDNQRLITTLEHLRDIGNTLIVVEHDEDTIRRADWLVDIGPRAGEFGGEVVYQGEPKGILDCEESLTGAYLSGRRTLGVPDTRREIDKERQLKVVGARENNLRGIDVKIPLGVLCCITGVSGSGKSTLVNQILAKVLANKLNRARQVPGRAKRVEGLEHLDKLVQVDQSPIGRTPRSNPATYTGVFDKVRNLFAETTEAKVRGYKPGRFSFNIKGGRCEACQGDGTLKIEMNFLPDVYVPCEVCDGQRYNRETLEVKYKGKNIAEVLGMPISEAADFFEPITSIHRYLATLVDVGLGYVRLGQAATTLSGGEAQRVKLAAELQKRSNGRTVYILDEPTTGLHFEDIRKLMMVIQGLVDKGNSVIIIEHNLDVIKAADWIVDMGPEGGSGGGTVVAEGTPEQVAEVAGSYTGQFLKELL

SEQ ID NO: 75 - DNA, 1446 bp, synthetic construct
  source 1..1446: mol_type = other DNA
atgcctaaacccctacccccagaaacccgacgcaagatcatcgatttcgatccgttcgcaccgaacagcccctcgatcgaagagttctgcagtcggctaaaaatatcgcggcgcagcttctacaacatccgcaaccgataccaacaagacgccaacgcagcactgcatccacgctccagcgccccaatcaccgcccggcgaacgtacgatgaatccatcaccagcaccttgctgtccatccgcgcacgcctgaaagcccaaggatgggagtacggcccgatctctattcgattcgaaggcatctccaccggggaactgactgcaccgattccatctgtttcaaccattgctcgtttgttacgcgccgcaggagctgttgaaagtaaccctaagaagcgaccgaagtcgtcggtggtgaggtttcaacgaggtcaagccatggaaatgtggcaaatagatggtttcatctacacactgcacgatactgatctgactcgggtaacgatctatcaaatccttgatgatgccactcggtttgatgtcggaacctgtgtctttcccgcgaatgaaaactcagtcgatgcccgaacagtgctagaacaagccattgctcatttcggtgccccgcatgaattactcagtgataacggctcagcgtttaaccggatgcggcaaggatacgtcggaagcttggaaagctatctcgcgacggtggggtgtttaagcattaccggcaagcctgggcatcctcaaacccaaggtaaaaacgaacgcagccaccgcacactatttcgtttccttcaagctcatcaaccacacacacttgaggaatgtgcgcactatattgaacagttccgcgatcattacaacaatcgtcgcccgcatcaggggttgccgaataatctcaccccggccgcggcctgggagattgtgggctgtgtggaacaacaacccccgattgatcccgtcgtgcttcaacagcaagccgatcactatgcccgtcgtcgaattgagaagcaatcagatgtcccgcttgttcggcaggaggaatctgttccggtgtctaagatgcagcagaccgagcaacgtcgacgggtacgtcgttttggtaaaaagccggtggatcctgatgtgtttacgtttgctgggaataatcagaaggtggtgttccaggggatgcgtatttctgttcctcgtacgatgagggacagggagttttatcggacggtgacggcaactgagcttggtttctgggatgcgataaccggggagcttgagttgtcgattccgttgctggttgtggcgattgcccggggtaagtcgtatgtcaattcttacaacattcgtggggtgtggatgcaacacccgacaccgttgtggcaacgcaaacgtgatgaggctgagaagcgatttaagtcgatagatccgggggatcttctgcgctag

SEQ ID NO: 76 - DNA, 1112 bp, synthetic construct
  source 1..1112: mol_type = other DNA
atgaccactgacatctacttcagccacaacaacccacacgacccatacgcccaccacaccaccgaactcaaccgcgacacccatcacctctgggtcaccctcaccaccgactccgacgacttcgacgcagactccttcaccaccgaagtcatccggatcaccggctactcccgccacgaagtcaacaacgggccttaacgccatggccgcgatgaccacctcccacacctacgcgcatccagacgctactactcttgagcatcgctactcgctcatcatgatcgcgtgcaaagcagacccaccctgtgggagactcgactgcgcatcacgacgctacacagtcacgcaggagtcatgatcatcctccaccctgctaacgcatcgccgcttgatcaagaactcgaaccgaccacgaggacccacaccgaagagactaggtcacgtcacaccaccgatgagccgactaggtcgcatcaaatcagcgcccacgcttgctcttcatgacatcatcaccactcaagacacagacacgaggacagctgctgaagcgctcatggccttcctgacagagaaaatccagttaaagatcaccaaatacctcttcaccccacacaatcacctgagcaggcatggtcaccagactacggtgacattgatcccgaagctacgacaatgccaccctcgtgtgcgccaaggacttagatgaggtcgctggagccacggagaagagctacaccccgagtgagaagatgaaagccctgatcagagctcgggatgggcattgccgcttcccagggtgttgcgtcccggccagtaaatgccaggtcgatcacattatcccgtgggcggagggcggcccgacagcggcgtggaacctgcagttgttgtgccagcggcatcacaatatgaaaaccgatggtcgctttactgctgatgctaatggattggcggagattagatggattgggccgatggatgtaccagcggtaactaggccgacgggtccgttggtgaaagcgatgccgcgggggatttggggtcaggtgttgagggatcggatccaggctaggtttgagcggatccgcgaccgcgccctcaacaaagaagactag

SEQ ID NO: 77 - DNA, 1938 bp, synthetic construct
  source 1..1938: mol_type = other DNA
gtggccaatctagattcagttcgccctggggtgcgggcagctcttcgacgtacccatacccaggtaaaaggtgtcgcgttgaccagggcattgattgcgcttgcagtaagcggagctttgcttagttccatgactccggcggtggcgcagccacagaatccggatgacgcagccattgcacaggcagaggaaaatgtttcggcgggcgatggggaagtcgcccgcctggcaggatctttgtccagcactgacgcggaaattaaccgcgtcgagctggaaatgggtgctctgcgtgaagaagtgaacaagtccctcgtggatttgcatgatgcgcaggcaatcgccgaacaggcccgccaagatgctcttgcagccaagaaggatctcgatgattctcaagcgcagatcgaagcagcccaagagcgccttgatgagatttcacgtgcagcgtatcgccaaaacggaacctccaaggggctttccggcatttcgggcaatggaaattctgaagatgcgctagatcgtcagacttacctgcgaaccagtgcggaaaagcagcaggcagctgttgaagagcttgatcgcctccgtacggaaaacgccaacaaggaatcggtgttgcgccaggcccgcatcgttgctgagcagcgtgaggcggaagccgtcgaaaagcaagtccagaccgaggctgcaattgccgcaaacagcgagcagctcaatgtcttgactaacaaccgcactaccttggttgcccagcgtgatgaggctgagcgcaacttggccatcgctcgtgcgcaggcggataatctgcaaggtcagcgtgctgagtacgaggaattccagcaggcagagcaggctcgcatccaggcggaagcggaagctcaggctgctgcggaggagaagcgtcgtgccgatgaggctgctgcacaggcagccgctgaagctcaagaggctgcccagcaagctcaggcagcggaggaagcccaagctgcgcaagcagctgaggcagcacaggcacaagcaactcaagctgcagaaacccaagctgcagaaacccaagctgcagaaacccaagctgcagaaacccaagctgcacaagccgcgcaagctcaggcagaagcgaatgatcgtgccgccgcgcaacagcgtgctgcagaggctcaagcagcagcggaacaggcgcaacgtgaggctgacgctcaggcggccaacgatgcccaagctcaggtactgcgtgaacaggcgctcactgcagcctccatcgctgcggctgctctaattgcggcgagccagtccagccatgccactactcaaaatccttacccaactgatgaagacgcggatccgaccgatattgcggacatccaaggcccaacgcagccaggtacgggtgagtctggagattcccagaacgactccagcgacaatgattccacaggcaacgattccacaggctctgactcttcagattcagattcctccggcaacgattcttcagaggttatttccggcgatcgttccgctcagattgagactgtgattgcgcgcgccatgagccagttgggtgtgcagtacgcatggggtggcggtaacgctaatggcccaactctgggtatccgtgacggtggcgtggcggactcttacggcgattacaacaaggttggcttcgactgctctggactgaccttgtatgcgtttgcgggtgtgggaatttcacttcctcactacacgggctaccagtaccagcacggcaccaaggtgtcgccttctgagatgcaacgtggcgatctgatcttctatggtccgggagcgtctcagcacgtggcaatttacctcggtgatggtcagatgattgaggctccgaattcgggttctgtcgtgaagatttctcctgttcgctggagcggaatgaccgagagcgtggtacgcctcatttag

SEQ ID NO: 78 - DNA, 612 bp, synthetic construct
  source 1..612: mol_type = other DNA
atgacgcagagcctgagagacgccaagcgggagtcgacccggcgagcgctcgccgagaccacctaccggatggtgcgtgcccgcggtttcgaccaggtgaccatcgacgagatcaccaccgaggtcaacgtctcccgccgtaccttctccaattacttcgccaacaaagaggaggcggtcgccttcgtgccggtcgaccgcatccggacggaactggagaagtgggaggcgccggcgggcatcgacgcggcggctgccgtgcgttccgtcgtcgcccacctgctcgccagcgggctgccgatgatgctcgccgagctcggtcgcctgggccgccgtcaccccccgttcggcccccacagcagggaggtccagtgggcggtgtgggacgcggtccgggaaaggctccacgaggtgctgcacatcgatgccccccgtgaccgccgtaacctcgcgatgctgctcggcgcgctctacggcatcgtgtcgacgcagctcgctgacctggatctgggcgacgaggggccgggccccgaggtgttcctggcgctgcaggagagcgtgggggaggtgttcacgctgttcgaaccggccctgcgccggatcgggcaatga

SEQ ID NO: 79 - DNA, 1446 bp, synthetic construct
  source 1..1446: mol_type = other DNA
atgcctaaacccctacccccagaaacccgacgcaagatcatcgatttcgatccgttcgcaccgaacagcccctcgatcgaagagttctgcagtcggctaaaaatatcgcggcgcagcttctacaacatccgcaaccgataccaacaagacgccaacgcagcactgcatccacgctccagcgccccgatcaccgcccggcgaacgtacgatgaatccatcaccagcaccttgctgtccatccgcgcacgcctgaaagcccaaggatgggagtacggcccgatctctattcgattcgaaggcatctccaccggggaactgactgcaccgattccatctgtttcaaccattgctcgtttgttacgcgccgcaggagctgttgaaagtaaccctaagaagcgaccgaagtcgtcggtggtgaggtttcaacgaggtcaagccatggaaatgtggcaaatagatggtttcatctacacactgcacgatactgatctgactcgggtcacgatctatcaaatccttgatgatgccactcggtttgatgtcggaacctgtgtctttcccgcgaatgaaaactcagtcgatgcccgaacagtgctagaacaagccattgctcatttcggtgccccgcatgaattactcagtgataacggctcagcgtttaaccggatgcggcaaggatacgtcggaagcttggaaagctatctcgcgacggtggggtgtttaagcattaccggcaagcctgggcatcctcaaacccaaggtaaaaacgaacgcagccaccgcacactatttcgtttccttcaagctcatcaaccacacacacttgaggaatgtgcgcactatattgaacagttccgcgatcattacaacaatcgtcgcccgcatcaggggttgccgaataatctcaccccggccgcggcctgggagattgtgggctgtgtggaacaacaacccccgattgatcccgtcgtgcttcaacagcaagccgatcactatgcccgtcgtcgaattgagaagcaatcagatgtcccgcttgttcggcaggaggaatctgttccggtgtctaagatgcagcagaccgagcaacgtcgacgggtacgtcgttttggtaaaaagccggtggatcctgatgtgtttacgtttgctgggaataatcagaaggtggtgttccaggggatgcgtatttctgttcctcgtacgatgagggacagggagttttatcggacggtgacggcaactgagcttggtttctgggatgcgataaccggggagcttgagttgtcgattccgttgccggttgtggcgattgcccggggtaagtcgtatgtcaattcttacaacattcgtggggtgtggatgcaacacccgacaccgttgtggcaacgcaaacgtgatgaggctgagaagcgattcaagtcgatagatccgggggatcttctgcgctag

SEQ ID NO: 80 - DNA, 2850 bp, synthetic construct
  source 1..2850: mol_type = other DNA
ttggctgatcgcctcgtagtgcgcggagcgcgtgaacacaacctaaaaggcgtggatattgatctgccacgcgactcgatggtggtgttcaccggcctgtcaggttccggtaaatcatcactggcctttgacaccatctttgcggaaggccagcgccgttacgtggagtcgttgtccagttacgcccgcatgttcttggggcagatggacaagccggacgtggatttgattgatggattatccccagcggtctccattgaccaaaagtccaccaaccgcaaccctcggtccaccgtcggtaccatcacggaagtctatgactacctgcgtcttctgtatgcccgcgctggtaccgcacactgcccagtgtgtgatgcccgcgtggagcgtcaaaccccgcagcagatggtggaccagatccttggcatggaggagggactgaagttccaaatccttgcgcctgtggtgcgtacccgtaaaggtgagttcgttgatcttttcgcagatcttgcatcccaaggttattcccgcgtgcgggttgatggggaagtgcaccagctctcggatcctccaaagctagaaaagcagatcaagcacgatattgatgttgtggttgaccgtctgcaggtaaaagccagccaaaagcagcgcctgacagactctatggaaaccgcacttcgcctggccgatggcgtggctgtgctggagttcgttggcctggaggaagatgatccgaataggcttcgtcgattctctgaaaagatgagctgccctaacggtcacgcgttgacggttgatgagctggagcctcgtgctttttccttcaactctccttatggcgcgtgtcctgcctgtgatggcttgggtgtgcgcaccgaagttgatattgatctgatcatcccagatccagatgcacctgcaactaaagcggttcagccctggaactccagcccaaaccactcttactttgaaaagctcattgaaggcctggcgaaagccctcggatttgatccggaaactccgtacagtgagctcaccgcagctcaaaagaaggctctggtctatggatcgaaggaagaagtaagcgttcgatacaagaaccgctacggacgcgtgcgttcttggactgcgccttttgaaggtgtcatgggctactttgatcgcaagttggagcagactgattccgaaacccaaaaagaccgactgttgggctacacccgtgaagtgccctgcccaacctgtaaaggcgcacgcctcaagccggaaatcttggccgtacgcctagactccggaagccatggagcgttgtccattgctggactaaccgcgctgtcggtgcatgaagcattcgagtttttggataacctcacactgggcaagcgcgaggaaatgatcgcgggagctgtgctgagggaaattcacgcccgcctgaaattcttgcttgacgtgggcctttcctacctcacccttgatcgcgccgcaggcaccctgtctggtggtgaagcgcagcgtatccgcctggctactcaaattggttccggtctggctggtgtgctctacgtcttggatgagccatccattggtctgcaccaacgtgacaaccagcgcttaatcactacccttgagcatctccgagatatcggaaacacactcattgttgtggaacacgatgaagacaccatcaggcgcgcagattggctcgtggatattggtcctcgagctggtgaatttggtggtgaagtggtctaccaaggtgagccgaagggcattttggactgcgaagaatccctcacaggtgcttacttgtctggtcgtcgaaccctgggtgttcctgatactcgccgtgagatcgacaaagagcgacagctcaaggtggttggtgctagggaaaacaacctgcggggcatcgatgtgaaaatcccactgggtgtgctgtgctgcatcactggtgtgtcgggatctggtaaatccacgctggtcaatcagattttggccaaggttctggccaacaaactcaaccgcgcacgccaagtgcctggtcgcgcaaagcgggtggaaggcctcgagcacttggataagttggtccaggtggatcagtcgccaattggtcgtactccacgttcaaacccagcgacgtacacgggtgtgtttgataaagtccgtaacctttttgccgagaccactgaagcgaaggtccgcggttacaagcctggccgcttctccttcaatattaagggtggacgctgcgaagcatgtcagggcgatggcacgctgaagatcgaaatgaacttcctgcccgacgtgtatgttccgtgtgaagtctgtgatggtcagcgctacaaccgcgagaccctcgaggtgaagtacaagggcaaaaacatcgctgaagtattgggcatgccgatctctgaggctgcggacttctttgagcccatcacctcaattcaccgatacctagcaacgctggttgatgtcggccttggctatgtccgtttgggccaggcagcaacaaccttgtctggtggtgaagcccagcgtgtgaaacttgccgctgagctgcagaagcgttccaacggtcgcaccgtttacatcctcgatgagccaactactggtttgcactttgaagatattcgcaaactcatgatggtgatccaaggcctggtggacaagggtaactccgtgatcatcatcgagcacaacctcgacgtgatcaaggctgccgactggatcgtggacatgggtccagaaggcggaagcggcggtggaactgtggtcgctgaaggaaccccagagcaagttgctgaagttgcgggttcctacaccggccaattccttaaagagttgttgtag

SEQ ID NO: 81 - DNA, 5802 bp, synthetic construct
  source 1..5802: mol_type = other DNA
gttcgcttgctgtccataaaaccgcccagtctagctatcgccatgtaagcccactgcaagctacctgctttctctttgcgcttgcgttttcccttgtccagatagcccagtagctgacattcatccggggtcagcaccgtttctgcggactggctttctacgtgttccgcttcctttagcagcccttgcgccctgagtgcttgcggcagcgtgaagctagcttttatcgccattcgccattcaggctgcgcaactgttgggaagggcgatcggtgcgggcctcttcgctattacgccagctggcgaaagggggatgtgctgcaaggcgattaagttgggtaacgccagggttttcccagtcacgacgttgtaaaacgacggccagtgaattcgagctcggtacccggggatcctctagagtcgacctgcaggcatgcaagcttggcgtaatcatggtcatagctgtttcctgtgtgaaattgttatccgctcacaattccacacaacatacgagccggaagcataaagtgtaaagcctggggtgcctaatgagtgagctaactcacattaattgcgttgcgctcactgcccgctttccagtcgggaaacctgtcgtgccagctgcattaatgaatcggccaacgcgcggggagaggcggtttgcgtattgggcgctcttccgcttcctcgctcactgactcgctgcgctcggtcgttcggctgcggcgagcggtatcagctcactcaaaggcggtaatacggttatccacagaatcaggggataacgcaggaaagaacatgtgagcaaaaggccagcaaaaggccaggaaccgtaaaaaggccgcgttgctggcgtttttccataggctccgcccccctgacgagcatcacaaaaatcgacgctcaagtcagaggtggcgaaacccgacaggactataaagataccaggcgtttccccctggaagctccctcgtgcgctctcctgttccgaccctgccgcttaccggatacctgtccgcctttctcccttcgggaagcgtggcgctttctcaatgctcacgctgtaggtatctcagttcggtgtaggtcgttcgctccaagctgggctgtgtgcacgaaccccccgttcagcccgaccgctgcgccttatccggtaactatcgtcttgagtccaacccggtaagacacgacttatcgccactggcagcagccactggtaacaggattagcagagcgaggtatgtaggcggtgctacagagttcttgaagtggtggcctaactacggctacactagaaggacagtatttggtatctgcgctctgctgaagccagttaccttcggaaaaagagttggtagctcttgatccggcaaacaaaccaccgctggtagcggtggtttttttgtttgcaagcagcagattacgcgcagaaaaaaaggatctcaagaagatcctttgatcttttctacggggtctgacgctcagtggaacgaaaactcacgttaagggattttggtcatgagattatcaaaaaggatcttcacctagatccttttggggtgggcgaagaactccagcatgagatccccgcgctggaggatcatccagccctgatagaaacagaagccactggagcacctcaaaaacaccatcatacactaaatcagtaagttggcagcatcacccgacgcactttgcgccgaataaatacctgtgacggaagatcacttcgcagaataaataaatcctggtgtccctgttgataccgggaagccctgggccaacttttggcgaaaatgagacgttgatcggcacgtaagaggttccaactttcaccataatgaaataagatcactaccgggcgtattttttgagttatcgagattttcaggagctgatagaaacagaagccactggagcacctcaaaaacaccatcatacactaaatcagtaagttggcagcatcacccgacgcactttgcgccgaataaatacctgtgacggaagatcacttcgcagaataaataaatcctggtgtccctgttgataccgggaagccctgggccaacttttggcgaaaatgagacgttgatcggcacgtaagaggttccaactttcaccataatgaaataagatcactaccgggcgtattttttgagttatcgagattttcaggagctctttggcatcgtctctcgcctgtcccctcagttcagtaatttcctgcatttgcctgtttccagtcggtagatattccacaaaacagcagggaagcagcgcttttccgctgcataaccctgcttcggggtcattatagcgattttttcggtatatccatcctttttcgcacgatatacaggattttgccaaagggttcgtgtagactttccttggtgtatccaacggcgtcagccgggcaggataggtgaagtaggcccacccgcgagcgggtgttccttcttcactgtcccttattcgcacctggcggtgctcaacgggaatcctgctctgcgaggctggccggctaccgccggcgtaacagatgagggcaagcggatggctgatgaaaccaagccaaccaggaagggcagcccacctatcaaggtgtactgccttccagacgaacgaagagcgattgaggaaaaggcggcggcggccggcatgagcctgtcggcctacctgctggccgtcggccagggctacaaaatcacgggcgtcgtggactatgagcacgtccgcgagggcgtcccggaaaacgattccgaagcccaacctttcatagaaggcggcggtggaatcgaaatctcgtgatggcaggttgggcgtcgcttggtcggtcatttcgaaaaaggttaggaatacggttagccatttgcctgcttttatatagttcatatgggattcacctttatgttgataagaaataaaagaaaatgccaataggatatcggcattttcttttgcgtttttatttgttaactgttaattgtccttgttcaaggatgctgtctttgacaacagatgttttcttgcctttgatgttcagcaggaagctcggcgcaaacgttgattgtttgtctgcgtagaatcctctgtttgtcatatagcttgtaatcacgacattgtttcctttcgcttgaggtacagcgaagtgtgagtaagtaaaggttacatcgttaggcggatcaagatccatttttaacacaaggccagttttgttcagcggcttgtatgggccagttaaagaattagaaacataaccaagcatgtaaatatcgttagacgtaatgccgtcaatcgtcatttttgatccgcgggagtcagtgaacaggtaccatttgccgttcattttaaagacgttcgcgcgttcaatttcatctgttactgtgttagatgcaatcagcggtttcatcacttttttcagtgtgtaatcatcgtttagctcaatcataccgagagcgccgtttgctaactcagccgtgcgttttttatcgctttgcagaagtttttgactttcttgacggaagaatgatgtgcttttgccatagtatgctttgttaaataaagattcttcgccttggtagccatcttcagttccagtgtttgcttcaaatactaagtatttgtggcctttatcttctacgtagtgaggatctctcagcgtatggttgtcgcctgagctgtagttgccttcatcgatgaactgctgtacattttgatacgtttttccgtcaccgtcaaagattgatttataatcctctacaccgttgatgttcaaagagctgtctgatgctgatacgttaacttgtgcagttgtcagtgtttgtttgccgtaatgtttaccggagaaatcagtgtagaataaacggatttttccgtcagatgtaaatgtggctgaacctgaccattcttgtgtttggtcttttaggatagaatcatttgcatcgaatttgtcgctgtctttaaagacgcggccagcgtttttccagctgtcaatagaagtttcgccgactttttgatagaacatgtaaatcgatgtgtcatccgcatttttaggatctccggctaatgcaaagacgatgtggtagccgtgatagtttgcgacagtgccgtcagcgttttgtaatggccagctgtcccaaacgtccaggccttttgcagaagagatatttttaattgtggacgaatcaaattcagaaacttgatatttttcatttttttgctgttcagggatttgcagcatatcatggcgtgtaatatgggaaatgccgtatgtttccttatatggcttttggttcgtttctttcgcaaacgcttgagttgcgcctcctgccagcagtgcggtagtaaaggttaatactgttgcttgttttgcaaactttttgatgttcatcgttcatgtctccttttttatgtactgtgttagcggtctgcttcttccagccctcctgtttgaagatggcaagttagttacgcacaataaaaaaagacctaaaatatgtaaggggtgacgccaaagtatacactttgccctttacacattttaggtcttgcctgctttatcagtaacaaacccgcgcgatttacttttcgacctcattctattagactctcgtttggattgcaactggtctattttcctcttttgtttgatagaaaatcataaaaggatttgcagactacgggcctaaagaactaaaaaatctatctgtttcttttcattctctgtattttttatagtttctgttgcatgggcataaagttgcctttttaatcacaattcagaaaatatcataatatctcatttcactaaataatagtgaacggcaggtatatgtgatgggttaaaaaggatcaccccagagtcccgctcagaagaactcgtcaagaaggcgatagaaggcgatgcgctgcgaatcgggagcggcgataccgtaaagcacgaggaagcggtcagcccattcgccgccaagctcttcagcaatatcacgggtagccaacgctatgtcctgatagcggtccgccacacccagccggccacagtcgatgaatccagaaaagcggccattttccaccatgatattcggcaagcaggcatcgccatgggtcacgacgagatcctcgccgtcgggcatccgcgccttgagcctggcgaacagttcggctggcgcgagcccctgatgctcttcgtccagatcatcctgatcgacaagaccggcttccatccgagtacgtgctcgctcgatgcgatgtttcgcttggtggtcgaatgggcaggtagccggatcaagcgtatgcagccgccgcattgcatcagccatgatggatactttctcggcaggagcaaggtgagatgacaggagatcctgccccggcacttcgcccaatagcagccagtcccttcccgcttcagtgacaacgtcgagacagctgcgcaaggaacgcccgtcgtggccagccacgatagccgcgctgcctcgtcttggagttcattcagggcaccggacaggtcggtcttgacaaaaagaaccgggcgcccctgcgctgacagccggaacacggcggcatcagagcagccgattgtctgttgtgcccagtcatagccgaatagcctctccacccaagcggccggagaacctgcgtgcaatccatcttgttcaatcatgcgaaacgatcctcatcctgtctcttgatcagatcttgatcccctgcgccatcagatccttggcggcaagaaagccatccagtttactttgcagggcttcccaaccttaccagagggcgccccagctggcaattccg